European Patent Application EP 4 278 900 A1, published November 22, 2023. Title: Method for preparing a pet food. Applicant: Paleo B.V. The sequence listing filed with the application follows.

SEQUENCE LISTING (14 sequences)

SEQ ID NO: 1 - protein, 154 aa, PRT
  Rat myoglobin
MGLSDGEWQMVLNIWGKVEGDLAGHGQEVLISLFKAHPETLEKFDKFKNLKSEEEMKSSEDLKKHGCTVLTALGTILKKKGQHAAEIQPLAQSHATKHKIPVKYLEFISEVIIQVLKKRYSGDFGADAQGAMSKALELFRNDIAAKYKELGFQG

SEQ ID NO: 2 - protein, 154 aa, PRT
  Rabbit myoglobin
MGLSDAEWQLVLNVWGKVEADLAGHGQEVLIRLFHTHPETLEKFDKFKHLKSEDEMKASEDLKKHGNTVLTALGAILKKKGHHEAEIKPLAQSHATKHKIPVKYLEFISEAIIHVLHSKHPGDFGADAQAAMSKALELFRNDIAAQYKELGFQG

SEQ ID NO: 3 - protein, 154 aa, PRT
  Mouse myoglobin
MGLSDGEWQLVLNVWGKVEADLAGHGQEVLIGLFKTHPETLDKFDKFKNLKSEEDMKGSEDLKKHGCTVLTALGTILKKKGQHAAEIQPLAQSHATKHKIPVKYLEFISEIIIEVLKKRHSGDFGADAQGAMSKALELFRNDIAAKYKELGFQG

SEQ ID NO: 4 - protein, 154 aa, PRT
  Steppe mammoth myoglobin
MGLSDGEWELVLKTWGKVEADIPGHGLEVFVRLFTGHPETLEKFDKFKHLKTEGEMKASEDLKKQGVTVLTALGGILKKKGHHQAEIQPLAHSHATKHKIPIKYLEFISDAIIHVLQSKHPAEFGADAQGAMKKALELFRNDIAAKYKELGFQG

SEQ ID NO: 5 - protein, 154 aa, PRT
  Woolly mammoth myoglobin
MGLSDGEWELVLKTWGKVEADIPGHGLEVFVRLFTGHPETLEKFDKFKHLKTEGEMKASEDLKKQGVTVLTALGGILKKKGHHQAEIQPLAQSHATKHKIPIKYLEFISDAIIHVLQSKHPAEFGADAQGAMKKALELFRNDIAAKYKELGFQG

SEQ ID NO: 6 - protein, 147 aa, PRT
  Tuna myoglobin
MADFDAVLKCWGPVEADYTTMGGLVLTRLFKEHPETQKLFPKFAGIAQADIAGNAAISAHGATVLKKLGELLKAKGSHAAILKPLANSHATKHKIPINNFKLISEVLVKVMHEKAGLDAGQQTALRNVMGIIIADLEANYKELGFSG

SEQ ID NO: 7 - DNA, 462 bp, DNA
  Rat myoglobin coding nucleid acid
atgggcctgagcgatggcgaatggcagatggtgctgaacatttggggcaaagtggaaggcgatctggcgggccatggccaggaagtgctgattagcctgtttaaagcgcatccggaaaccctggaaaaatttgataaatttaaaaacctgaaaagcgaagaagaaatgaaaagcagcgaagatctgaaaaaacatggctgcaccgtgctgaccgcgctgggcaccattctgaaaaaaaaaggccagcatgcggcggaaattcagccgctggcgcagagccatgcgaccaaacataaaattccggtgaaatatctggaatttattagcgaagtgattattcaggtgctgaaaaaacgctatagcggcgattttggcgcggatgcgcagggcgcgatgagcaaagcgctggaactgtttcgcaacgatattgcggcgaaatataaagaactgggctttcagggc

SEQ ID NO: 8 - DNA, 462 bp, DNA
  Rabbit myoglobin coding nucleid acid
atgggcctgagcgatgcggaatggcagctggtgctgaacgtgtggggcaaagtggaagcggatctggcgggccatggccaggaagtgctgattcgcctgtttcatacccatccggaaaccctggaaaaatttgataaatttaaacatctgaaaagcgaagatgaaatgaaagcgagcgaagatctgaaaaaacatggcaacaccgtgctgaccgcgctgggcgcgattctgaaaaaaaaaggccatcatgaagcggaaattaaaccgctggcgcagagccatgcgaccaaacataaaattccggtgaaatatctggaatttattagcgaagcgattattcatgtgctgcatagcaaacatccgggcgattttggcgcggatgcgcaggcggcgatgagcaaagcgctggaactgtttcgcaacgatattgcggcgcagtataaagaactgggctttcagggc

SEQ ID NO: 9 - DNA, 462 bp, DNA
  Mouse myoglobin coding nucleid acid
atgggcctgagcgatggcgaatggcagctggtgctgaacgtgtggggcaaagtggaagcggatctggcgggccatggccaggaagtgctgattggcctgtttaaaacccatccggaaaccctggataaatttgataaatttaaaaacctgaaaagcgaagaagatatgaaaggcagcgaagatctgaaaaaacatggctgcaccgtgctgaccgcgctgggcaccattctgaaaaaaaaaggccagcatgcggcggaaattcagccgctggcgcagagccatgcgaccaaacataaaattccggtgaaatatctggaatttattagcgaaattattattgaagtgctgaaaaaacgccatagcggcgattttggcgcggatgcgcagggcgcgatgagcaaagcgctggaactgtttcgcaacgatattgcggcgaaatataaagaactgggctttcagggc

SEQ ID NO: 10 - DNA, 465 bp, DNA
  Steppe mammoth myoglobin coding nucleid acid
atgggactcagcgacggggaatgggagttggtgttgaaaacctgggggaaagtggaggctgacatcccgggccatgggctggaagtcttcgtcaggctcttcacaggtcatcccgagaccctggagaagttcgacaagtttaagcacctgaagacagagggcgagatgaaggcctccgaggacctgaagaagcaaggtgttactgtgctcactgccctggggggcatcctcaagaagaaagggcatcaccaggcggagattcagcccctggcccattctcatgccaccaagcacaagatccccatcaagtatctggagttcatctcggacgccatcatccacgttctgcaaagcaagcatcctgcggaatttggcgctgatgcccagggagccatgaaaaaggccttggagctgttccggaatgacattgcggccaagtataaggagctggggttccagggctag

SEQ ID NO: 11 - DNA, 465 bp, DNA
  Woolly mammoth myoglobin coding nucleid acid
atgggactcagcgacggggaatgggagttggtgttgaaaacctgggggaaagtggaggctgacatcccgggccatgggctggaagtcttcgtcaggctcttcacaggtcatcccgagaccctggagaagttcgacaagtttaagcacctgaagacagagggcgagatgaaggcctccgaggacctgaagaagcaaggtgttactgtgctcactgccctggggggcatcctcaagaagaaagggcatcaccaggcggagattcagcccctggcccagtctcatgccaccaagcacaagatccccatcaagtatctggagttcatctcggacgccatcatccacgttctgcaaagcaagcatcctgcggaatttggcgctgatgcccagggagccatgaaaaaggccttggagctgttccggaatgacattgcggccaagtataaggagctggggttccagggctag

SEQ ID NO: 12 - DNA, 444 bp, DNA
  Tuna myoglobin coding nucleid acid
atggctgactttgatgcagttctgaagtgttggggtccagtggaggcggactacaccaccattggaggcctggttctgacccgtttattcaaagagcaccctgagacccagaagctgttccccaaattcgctggcatcgcccaggctgacatagccggtaacgcagctgtttctgctcatggtgccactgtgctgaagaaacttggagagctgctgaaggccaaaggcagtcacgctgccatcctaaaaccactggcaaacagccatgccactaagcacaagattcccattaataacttcaagctgatttctgaggtccttgtgaaggtcatgcatgagaaggcaggactcgatgccggtgggcagacagccctgaggaacgtgatgggtatcatcatcgccgaccttgaggccaactacaaagagctgggcttctctggctga

SEQ ID NO: 13 - protein, 175 aa, PRT
  Woolly mammoth k-casein
MKGFLLVVNILLLPLFLAAEVQNQEESRCLEKDERWFCQKAVKYIPNDYVLKSYYRYEPNYNQFRAAVPINNPYLIYLYPAKQVAVRPHTQIQWQVPSNIYPSPSVPHTYLKPPFIIPPKKTQDKPIIPPTGTVASIEATVEPKVNTVVNAEASSEFIATNTPEATTVPVISPQI

SEQ ID NO: 14 - protein, 260 aa, PRT
  Woolly mammoth b-casein
MKVFILACLVAFALGRETVENLSSSEIRQFYSEQKPEGVKHEEQQREDEHQNKIQPLFQPQPLVYPFAEPIPYTVFPPNAIPLAQPIVVLPFPQPEVQLPEAKEITFPRQKLMSFLKSPVMPFFDPQPNLGTDLENLHLPLPLLQPLRHQLHQPLAQTPVLPLPLSLPKVLPVPQQVIPYPQRGRPIQNLLYEEPLLDPTRKIYPVAQPLAPVYNPVAYMIGIPCCSTLLTYLHQSSRSQYPIQNKLGYLIAMPKKVRPT